European Patent Specification EP 3 681 481 B1, published May 6, 2026. Title: COMPOSITIONS AND METHODS FOR PREVENTING AND TREATING HETEROTROPIC OSSIFICATION AND PATHOLOGIC CALCIFICATION. Applicant: Nostopharma, LLC. The sequence listing filed with the application follows.

SEQUENCE LISTING (4 sequences)

SEQ ID NO: 1 - DNA, 22 bp, Artificial Sequence
  Primer sequence
cacagcttctttgcagctcctt

SEQ ID NO: 2 - DNA, 19 bp, Artificial Sequence
  Primer Sequence
cgtcatccatggcgaactg

SEQ ID NO: 3 - DNA, 23 bp, Artificial Sequence
  Primer Sequence
cacgcgatgcaacaccactcagg

SEQ ID NO: 4 - DNA, 21 bp, Artificial Sequence
  Primer sequence
gcatgtccccgggctcaaaga